European Patent Specification EP 4 034 084 B1, published November 5, 2025. Title: COMPOSITIONS AND METHODS TO TREAT METASTATIC GASTROINTESTINAL CANCER. Applicant: Rockefeller University Tavazoie, Sohail Yamaguchi, Norihiro Tavazoie, Masoud. The sequence listing filed with the application follows.

SEQUENCE LISTING (10 sequences)

SEQ ID NO: 1 - DNA, 19 bp, artificial
  synthetic
aaggtgttcccattgaagg

SEQ ID NO: 2 - DNA, 20 bp, artificial
  synthetic
gaagttgtagccaaagaagg

SEQ ID NO: 3 - DNA, 20 bp, artificial
  synthetic
gaccagtcaacaggggacat

SEQ ID NO: 4 - DNA, 20 bp, artificial
  synthetic
cctgaccaaggaaagcaaag

SEQ ID NO: 5 - DNA, 21 bp, artificial
  synthetic
ctgcataacggtctggacttc

SEQ ID NO: 6 - DNA, 19 bp, artificial
  synthetic
cagcaactgcccgtactcc

SEQ ID NO: 7 - DNA, 20 bp, artificial
  synthetic
ggctgtattcccctccatcg

SEQ ID NO: 8 - DNA, 22 bp, artificial
  synthetic
ccagttggtaacaatgccatgt

SEQ ID NO: 9 - DNA, 20 bp, artificial
  synthetic
ccacgggagatgagcgtttc

SEQ ID NO: 10 - DNA, 19 bp, artificial
  synthetic
cagggaggtgaagcgaaca